European Patent Specification EP 3 880 692 B1, published January 3, 2024. Title: NOVEL TRIPLE-HELICAL POLYPEPTIDES LACKING BINDING AFFINITY FOR THE FC DOMAIN OF IMMUNOGLOBULIN AND USES THEREOF. Applicant: Navigo Proteins GmbH. The sequence listing filed with the application follows.

SEQUENCE LISTING (34 sequences)

SEQ ID NO: 1 - protein, 58 aa, Artificial Sequence
  PAdelFc (27+ with 10S, 13D, 14S, 31R, 35S)
IAAKFDEAQSAADSEILHLPNLTEEQRNAFRQSLSDDPSVSLEVLGEAQKLNDSQAPK

SEQ ID NO: 2 - protein, 58 aa, Artificial Sequence
  PAdelFc (27+ with 13D 31R)
IAAKFDEAQQAADYEILHLPNLTEEQRNAFRQSLRDDPSVSLEVLGEAQKLNDSQAPK

SEQ ID NO: 3 - protein, 58 aa, Artificial Sequence
  PAdelFc (27+ with 13D 31R 35S)
IAAKFDEAQQAADYEILHLPNLTEEQRNAFRQSLSDDPSVSLEVLGEAQKLNDSQAPK

SEQ ID NO: 4 - protein, 58 aa, Artificial Sequence
  PAdelFc (27+ with 10S 13D 31R)
IAAKFDEAQSAADYEILHLPNLTEEQRNAFRQSLRDDPSVSLEVLGEAQKLNDSQAPK

SEQ ID NO: 5 - protein, 58 aa, Artificial Sequence
  #PAdelFc (27+ with 10S 13D 31R 35S)
IAAKFDEAQSAADYEILHLPNLTEEQRNAFRQSLSDDPSVSLEVLGEAQKLNDSQAPK

SEQ ID NO: 6 - protein, 58 aa, Artificial Sequence
  PAdelFc (27+ with 13D 14S 31R)
IAAKFDEAQQAADSEILHLPNLTEEQRNAFRQSLRDDPSVSLEVLGEAQKLNDSQAPK

SEQ ID NO: 7 - protein, 58 aa, Artificial Sequence
  PAdelFc (27+ with 10S 13D 14S 31R)
IAAKFDEAQSAADSEILHLPNLTEEQRNAFRQSLRDDPSVSLEVLGEAQKLNDSQAPK

SEQ ID NO: 8 - protein, 58 aa, Artificial Sequence
  PAdelFc (27+ with 13D 14S 31R 35S)
IAAKFDEAQQAADSEILHLPNLTEEQRNAFRQSLSDDPSVSLEVLGEAQKLNDSQAPK

SEQ ID NO: 9 - protein, 58 aa, Artificial Sequence
  PAdelFc (27 with 10S, 13D, 14S, 31R, 35S)
NAAKFDEAQSSADSEILHLPNLTEEQRNAFRQSLSDDPSVSKEVLGEAQKLNDSQAPK

SEQ ID NO: 10 - protein, 58 aa, Artificial Sequence
  PAdelFc (14+ with 13D, 31R)
IAAKHDKDQQAADYEILHLPNLTEDQRNAFRQSLRDDPSVSLEILGEAKKLNDAQAPP

SEQ ID NO: 11 - protein, 58 aa, Artificial Sequence
  PAdelFc (14+ with 10S, 13D, 14S, 31R, 35S)
IAAKHDKDQSAADSEILHLPNLTEDQRNAFRQSLSDDPSVSLEILGEAKKLNDAQAPP

SEQ ID NO: 12 - protein, 58 aa, Artificial Sequence
  PAdelFc (50+ with 13D 31R)
IDAKFDEAQQAADYEILHLPNLTEDQRNAFRQSLRDDPSVSLSLLAEAKKLNDAQAPP

SEQ ID NO: 13 - protein, 58 aa, Artificial Sequence
  PAdelFc (50+ with 10S, 13D, 14S, 31R, 35S)
IDAKFDEAQSAADSEILHLPNLTEDQRNAFRQSLSDDPSVSLSLLAEAKKLNDAQAPP

SEQ ID NO: 14 - protein, 58 aa, Artificial Sequence
  PAdelFc (54+ with 13D 31R)
IDAQHDEDQQAADYEILHLPNLTEEQRNAFRQSLRDDPSQSLEILAEAKKLNESQAPK

SEQ ID NO: 15 - protein, 58 aa, Artificial Sequence
  PAdelFc (54+ with 10S, 13D, 14S, 31R, 35S)
IDAQHDEDQSAADSEILHLPNLTEEQRNAFRQSLSDDPSQSLEILAEAKKLNESQAPK

SEQ ID NO: 16 - protein, 58 aa, Artificial Sequence
  27+
IAAKFDEAQQAAFYEILHLPNLTEEQRNAFIQSLRDDPSVSLEVLGEAQKLNDSQAPK

SEQ ID NO: 17 - protein, 58 aa, Artificial Sequence
  27
NAAKFDEAQQSAFYEILHLPNLTEEQRNAFIQSLKDDPSVSKEVLGEAQKLNDSQAPK

SEQ ID NO: 18 - protein, 218 aa, Artificial Sequence
  IgG1 Fc region
PAPELLGGPSVFLFPPKPKDTLMISRTPEVTCVVVDVSHEDPEVKFNWYVDGVEVHNAKTKPREEQYNSTYRVVSVLTVLHQDWLNGKEYKCKVSNKALPAPIEKTISKAKGQPREPQVYTLPPSREEMTKNQVSLTCLVKGFYPSDIAVEWESNGQPENNYKTTPPVLDSDGSFFLYSKLTVDKSRWQQGNVFSCSVMHEALHNHYTQKSLSLSPGK

SEQ ID NO: 19 - protein, 218 aa, Artificial Sequence
  IgG1 Fc
PAPELLGGPSVFLFPPKPKDTLMISRTPEVTCVVVDVSHEDPEVKFNWYVDGVEVHNAKTKPREEQYNSTYRVVSVLTVLHQDWLNGKEYKCKVSNKALPAPIEKTISKAKGQPREPQVYTLPPSRDELTKNQVSLTCLVKGFYPSDIAVEWESNGQPENNYKTTPPVLDSDGSFFLYSKLTVDKSRWQQGNVFSCSVMHEALHNHYTQKSLSLSPGK

SEQ ID NO: 20 - protein, 58 aa, Artificial Sequence
  domain C
ADNKFNKEQQNAFYEILHLPNLTEEQRNGFIQSLKDDPSVSKEILAEAKKLNDAQAPK

SEQ ID NO: 21 - protein, 58 aa, Artificial Sequence
  domain A
ADNNFNKEQQNAFYEILNMPNLNEEQRNGFIQSLKDDPSQSANLLAEAKKLNESQAPK

SEQ ID NO: 22 - protein, 58 aa, Artificial Sequence [sequence omitted]

SEQ ID NO: 23 - protein, 58 aa, Artificial Sequence
  PAdelFc  (24+ 13D 31R)
IAAQHDKEQQAADYEILHLPNLTEDQRNAFRQSLRDDPSVSLEILGEAKKLNDAQAPK

SEQ ID NO: 24 - protein, 58 aa, Artificial Sequence
  PAdelFc (24+ 10S 13D 14S 31R 35S)
IAAQHDKEQSAADSEILHLPNLTEDQRNAFRQSLSDDPSVSLEILGEAKKLNDAQAPK

SEQ ID NO: 25 - protein, 58 aa, Artificial Sequence
  PAdelFc (26+ 13D 31R)
IAAQHDKDQQAADYEILHLPNLTEEQRNAFRQSLRDDPSVSLEILAEAKKLNDAQAPK

SEQ ID NO: 26 - protein, 58 aa, Artificial Sequence
  PAdelFc (26+ 10S 13D 14S 31R 35S)
IAAQHDKDQSAADSEILHLPNLTEEQRNAFRQSLSDDPSVSLEILAEAKKLNDAQAPK

SEQ ID NO: 27 - protein, 58 aa, Artificial Sequence
  PAdelFc (60+ 13D 31R)
IDAKFDEAAQAADYEILHLPNLTEDQRNAFRQSLRDDPSVSLALLAEAKKLNDAQAPP

SEQ ID NO: 28 - protein, 58 aa, Artificial Sequence
  PAdelFc (60+ with 10S, 13D, 14S, 31R, 35S)
IDAKFDEAASAADSEILHLPNLTEDQRNAFRQSLSDDPSVSLALLAEAKKLNDAQAPP

SEQ ID NO: 29 - protein, 58 aa, Artificial Sequence
  PAdelFc (59+ 13D 31R)
IDAKFDEAQQAADYEILHLPNLTEDQRNAFRQSLRDDPSVSLALLAEAKKLNDAQAPP

SEQ ID NO: 30 - protein, 58 aa, Artificial Sequence
  PAdelFc (59+ with 10S, 13D, 14S, 31R, 35S)
IDAKFDEAQSAADSEILHLPNLTEDQRNAFRQSLSDDPSVSLALLAEAKKLNDAQAPP

SEQ ID NO: 31 - protein, 58 aa, Artificial Sequence
  PA02
  Xaa (25)..(25): can be any amino acid except C, G, N, P
  Xaa (26)..(26): can be any amino acid except C, G, N, P
  Xaa (28)..(28): can be any amino acid except C, G, N, P
  Xaa (29)..(29): can be any amino acid except C, G, N, P
  Xaa (30)..(30): F, H, or Y
  Xaa (32)..(32): can be any amino acid except C, G, N, P
  Xaa (33)..(33): can be any amino acid except C, G, N, P
  Xaa (35)..(35): can be any amino acid except C, G, N, P
  Xaa (36)..(36): can be any amino acid except C, G, N, P
  Xaa (42)..(42): can be any amino acid except C, G, N, P
  Xaa (43)..(43): can be any amino acid except C, G, N, P
  Xaa (44)..(44): I, L, T, or V
  Xaa (46)..(46): can be any amino acid except C, G, N, P
  Xaa (47)..(47): can be any amino acid except C, G, N, P
  Xaa (50)..(50): can be any amino acid except C, G, N, P
  Xaa (54)..(54): can be any amino acid except C, G, N, P
IAAKFDEAQSAADSEILHLPNLTEXXRXXXRXXLXXDPSVSXXXLXXAQXLNDXQAPK

SEQ ID NO: 32 - protein, 58 aa, Artificial Sequence
  PA12
  Xaa (25)..(25): H, E, V, A, L, Y, W, K, I, Q, T, or R
  Xaa (29)..(29): H, E, V, A, L, Y, W, K, I, Q, T, or R
  Xaa (33)..(33): H, E, V, A, L, Y, W, K, I, Q, T, or R
  Xaa (36)..(36): H, E, V, A, L, Y, W, K, I, Q, T, or R
  Xaa (37)..(37): H, E, V, A, L, Y, W, K, I, Q, T, or R
  Xaa (43)..(43): H, E, V, A, L, Y, W, K, I, Q, T, or R
  Xaa (46)..(46): H, E, V, A, L, Y, W, K, I, Q, T, or R
  Xaa (47)..(47): H, E, V, A, L, Y, W, K, I, Q, T, or R
  Xaa (50)..(50): H, E, V, A, L, Y, W, K, I, Q, T, or R
  Xaa (51)..(51): H, E, V, A, L, Y, W, K, I, Q, T, or R
  Xaa (54)..(54): H, E, V, A, L, Y, W, K, I, Q, T, or R
IAAKFDEAQSAADSEILHLPNLTEXQRNXFRQXLSXXPSVSLXVLXXAQXXNDXQAPK

SEQ ID NO: 33 - protein, 58 aa, Artificial Sequence
  PA03
  Xaa (7)..(7): A, L, M, F, W, K, Q, E, S, V, I, Y, H, R, D, or T
  Xaa (8)..(8): A, L, M, F, W, K, Q, E, S, V, I, Y, H, R, D, or T
  Xaa (10)..(10): A, L, M, F, W, K, Q, E, S, V, I, Y, H, R, D, or T
  Xaa (11)..(11): A, L, M, F, W, K, Q, E, S, V, I, Y, H, R, D, or T
  Xaa (14)..(14): A, L, M, F, W, K, Q, E, S, V, I, Y, H, R, D, or T
  Xaa (15)..(15): A, L, M, F, W, K, Q, E, S, V, I, Y, H, R, D, or T
  Xaa (18)..(18): A, L, M, F, W, K, Q, E, S, V, I, Y, H, R, D, or T
  Xaa (20)..(20): A, L, M, F, W, K, Q, E, S, V, I, Y, H, R, D, or T
  Xaa (42)..(42): A, L, M, F, W, K, Q, E, S, V, I, Y, H, R, D, or T
  Xaa (43)..(43): A, L, M, F, W, K, Q, E, S, V, I, Y, H, R, D, or T
  Xaa (46)..(46): A, L, M, F, W, K, Q, E, S, V, I, Y, H, R, D, or T
  Xaa (47)..(47): A, L, M, F, W, K, Q, E, S, V, I, Y, H, R, D, or T
  Xaa (49)..(49): A, L, M, F, W, K, Q, E, S, V, I, Y, H, R, D, or T
  Xaa (50)..(50): A, L, M, F, W, K, Q, E, S, V, I, Y, H, R, D, or T
  Xaa (53)..(53): A, L, M, F, W, K, Q, E, S, V, I, Y, H, R, D, or T
  Xaa (54)..(54): A, L, M, F, W, K, Q, E, S, V, I, Y, H, R, D, or T
IAAKFDXXQXXADXXILXLXNLTEEQRNAFRQSLSDDPSVSXXVLXXAXXLNXXQAPK

SEQ ID NO: 34 - protein, 58 aa, Artificial Sequence
  PA13
  Xaa (7)..(7): H, E, V, A, L, Y, W, K, I, Q, T, or R
  Xaa (8)..(8): H, E, V, A, L, Y, W, K, I, Q, T, or R
  Xaa (11)..(11): H, E, V, A, L, Y, W, K, I, Q, T, or R
  Xaa (14)..(14): H, E, V, A, L, Y, W, K, I, Q, T, or R
  Xaa (15)..(15): H, E, V, A, L, Y, W, K, I, Q, T, or R
  Xaa (18)..(18): H, E, V, A, L, Y, W, K, I, Q, T, or R
  Xaa (42)..(42): H, E, V, A, L, Y, W, K, I, Q, T, or R
  Xaa (46)..(46): H, E, V, A, L, Y, W, K, I, Q, T, or R
  Xaa (49)..(49): H, E, V, A, L, Y, W, K, I, Q, T, or R
  Xaa (50)..(50): H, E, V, A, L, Y, W, K, I, Q, T, or R
  Xaa (53)..(53): H, E, V, A, L, Y, W, K, I, Q, T, or R
IAAKFDXXQSXADXXILXLPNLTEEQRNAFRQSLSDDPSVSXEVLXEAXXLNXSQAPK